European Patent Application EP 4 403 630 A1, published July 24, 2024. Title: 耐高温甘露聚糖酶突变体. Applicant: 青岛蔚蓝生物集团有限公司. Application CN. The sequence listing filed with the application follows.

SEQUENCE LISTING (2 sequences)

SEQ ID NO: 1 - protein, 362 aa, synthetic construct
LPKASPAPSTSSSAASTSFASTSGLQFTIDGETGYFAGTNSYWIGFLTDNADVDLVMGHLKSSGLKILRVWGFNDVTSQPSSGTVWYQLHQDGKSTINTGADGLQRLDYVVSSAEQHDIKLIINFVNYWTDYGGMSAYVSAYGGSGETDFYTSDTMQSAYQTYIKTVVERYSNSSAVFAWELANEPRCPSCDTSVLYNWIEKTSKFIKGLDADRMVCIGDEGFGLNIDSDGSYPYQFSEGLNFTMNLGIDTIDFGTLHLYPDSWGTSDDWGNGWITAHGAACKAAGKPCLLEEYGVTSNHCSVEGSWQKTALSTTGVGADLFWQYGDDLSTGKSPDDGNTIYYGTSDYQCLVTDHVAAIDSA

SEQ ID NO: 2 - DNA, 1089 bp, synthetic construct
  source 1..1089: mol_type = other DNA
ctgccgaaagcctcccctgcaccgagcaccagcagcagtgctgcctccacctccttcgccagcacctccggcctccaattcaccattgatggcgaaactggctacttcgccggaacgaacagctactggatcggtttcctcactgacaacgcggacgtcgacctcgtcatgggccacctgaagtcgtccggcctcaagatcctccgcgtgtggggcttcaacgatgtcacctcgcagccctcctccggcacagtctggtaccaactgcaccaggacggcaaatcgacaatcaacacgggtgccgacggtctccagcgcctcgactacgtcgtctcgtctgccgaacagcacgacatcaaactcatcatcaacttcgtcaactactggaccgattacggtggtatgtctgcgtacgtgagcgcgtatggcggatccggcgagacggatttctataccagtgataccatgcagagtgcctatcagacatatatcaagacggtcgtggagcggtacagtaactcctcggcggtgtttgcgtgggagttggcgaatgagccgagatgtccgagttgcgatacttctgtgttgtataactggattgagaagacgagtaagtttattaaggggttggatgcggatcgtatggtttgtattggtgatgagggcttcggtctcaacatcgactcggacggcagctacccttatcaattctccgagggcttgaactttacgatgaacctcggtatcgatactattgactttggtaccctccacttgtaccctgatagctggggcacctccgacgactggggcaacggctggatcaccgcccacggcgcagcctgcaaagcggccggcaagccatgtctcctggaggaatacggagtcacctcgaaccactgcagtgtggagggctcgtggcagaagacagcgctcagcacaacgggcgtcggcgcggatctgttctggcagtatggtgatgatttgagtaccgggaagtcgccggatgatgggaatactatctactatgggactagtgattatcagtgcctggtgacggatcatgttgctgctattgatagcgcctaa